European Patent Application EP 4 524 238 A1, published March 19, 2025. Title: 혈액 적합성을 갖는 혈관 내 이식용 세포, 이의 제조방법 및 용도. Applicant: 주식회사 툴젠. Application KR PCT230312, filed May 11, 2023. The sequence listing filed with the application follows.

SEQUENCE LISTING (3 sequences)

SEQ ID NO: 1 - DNA, 23 bp, Homo sapiens
  source 1..23: mol_type = genomic DNA
tctggggagttctcatacagagg

SEQ ID NO: 2 - DNA, 20 bp, synthetic construct
  source 1..20: mol_type = other DNA
gcactaagtcaggagattgg

SEQ ID NO: 3 - DNA, 20 bp, synthetic construct
  source 1..20: mol_type = other DNA
gttcagacgtttctaacaag